European Patent Specification EP 3 530 735 B1, published September 10, 2025. Title: Recombinant silk from bag worm. Applicant: National Agriculture and Food Research Organization. The sequence listing filed with the application follows.

SEQUENCE LISTING (33 sequences)

SEQ ID NO: 1 - protein, 13 aa, Eumeta japonica
GAGAGAGSGAGAG

SEQ ID NO: 2 - DNA, 39 bp, Eumeta japonica
ggagccggagcaggtgccggttcaggcgccggtgctgga

SEQ ID NO: 3 - DNA, 39 bp, Eumeta japonica
ggtgccggagcaggagctggatcaggtgcaggagcaggt

SEQ ID NO: 4 - DNA, 39 bp, Eumeta japonica
ggtgcgggcgctggagcaggttccggagcaggagcaggt

SEQ ID NO: 5 - protein, 140 aa, Eumeta japonica
VVYVSAGGAGAGAGSGAGAGSGAGAGAGSGAGAGGAGAAAGAGAGAGSGAGSGSGAGAGAGSGAGAGSGAGAGAGAGSGAAGGAGAGAGAGAAAAAAAAAEAAAAAAAAAAAAGSGAGAGGAGGYGAGAGAGAGAGAGGA

SEQ ID NO: 6 - DNA, 420 bp, Eumeta japonica
gtcgtctacgtaagtgctggaggagccggagcaggtgccggttcaggcgccggtgctggatcgggtgccggagcaggagctggatcaggtgcaggagcaggtggagcaggagccgcagccggagctggtgctggtgctggttcaggtgcaggatccggttcaggtgcgggcgctggagcaggttccggagcaggagcaggttccggtgctggtgcaggagcaggagctggttcaggtgcagcaggtggagcaggagctggcgctggcgctggcgctgcagccgcagccgcagcagcagcagaagcggcagccgcagctgccgccgccgctgccgccgcaggtagtggagcaggcgctggaggagccggaggctacggagcgggagctggagcaggtgccggtgcaggtgctggcggcgca

SEQ ID NO: 7 - protein, 308 aa, Eumeta japonica
IAASVGAGVGAASVAGAGTGAGSGAAGGAGAGADAGAAAAAAAAAQAAAADAAAAGSGAGAGRVGAYGPYGGLASAGAGGAGGAGGAGGYSGASVVYVSAGGAGAGAGSGAGAGSGAGAGAGSGAGAGGAGAAAGAGAGAGSGAGSGSGAGAGAGSGAGAGSGAGAGAGAGSGAAGGAGAGAGAGAAAAAAAAAEAAAAAAAAAAAAGSGAGAGGAGGYGAGAGAGAGAGAGGASGGYGSYGSGVAAGAGAGAGVGGSRGAGVGAGVGAGYGSALNSGAGAGAGAGAGAGGAAGAGAGAGAGAGAGAG

SEQ ID NO: 8 - DNA, 924 bp, Eumeta japonica
atagcagccagtgtaggtgcgggcgttggagcagcttccgttgctggtgcaggaacaggagctggctcaggtgcagctggtggagcaggagcaggtgctgacgctggcgctgcagccgccgctgcggcagcagcacaagcagcagccgcagatgctgccgccgcaggtagtggcgctggtgctggacgagtcggagcttacggaccctacggaggtttagcaagcgctggtgctggtggtgctggcggagccggtggtgcaggtggatacagtggtgcaagtgtcgtctacgtaagtgctggaggagccggagcaggtgccggttcaggcgccggtgctggatcgggtgccggagcaggagctggatcaggtgcaggagcaggtggagcaggagccgcagccggagctggtgctggtgctggttcaggtgcaggatccggttcaggtgcgggcgctggagcaggttccggagcaggagcaggttccggtgctggtgcaggagcaggagctggttcaggtgcagcaggtggagcaggagctggcgctggcgctggcgctgcagccgcagccgcagcagcagcagaagcggcagccgcagctgctgccgccgctgccgccgcaggtagtggagcaggcgctggaggagccggaggctacggagcgggagctggagcaggtgccggtgcaggtgctggcggcgcatctggaggctacggttcttacggatcgggagttgcagcaggtgccggtgcaggagctggtgttggtggtagcaggggagcaggtgttggcgctggtgttggtgctggttatggctccgcattgaattcaggagccggtgccggagcaggtgctggtgctggagctggtggtgctgcaggagctggtgctggtgcaggagcaggagctggcgctggagctgga

SEQ ID NO: 9 - protein, 530 aa, Artificial
  chimeric protein
MRVKTFVILCCALQYVAYTNANINDFDEDYFGSDVTVQSSNTTDEIIRDASGAVIEEQITTKKMQRKNKNHGILGKNEKMIKTFVITTDSDGNESIVEEDVLMKTLSDGTVAQSYVAADAGAYSQSGPYVSNSGYSTHQGYTSDFSTSAAVGAGSIAASVGAGVGAASVAGAGTGAGSGAAGGAGAGADAGAAAAAAAAAQAAAADAAAAGSGAGAGRVGAYGPYGGLASAGAGGAGGAGGAGGYSGASVVYVSAGGAGAGAGSGAGAGSGAGAGAGSGAGAGGAGAAAGAGAGAGSGAGSGSGAGAGAGSGAGAGSGAGAGAGAGSGAAGGAGAGAGAGAAAAAAAAAEAAAAAAAAAAAAGSGAGAGGAGGYGAGAGAGAGAGAGGASGGYGSYGSGVAAGAGAGAGVGGSRGAGVGAGVGAGYGSALNSGAGAGAGAGAGAGGAAGAGAGAGAGAGAGAGVDSVSYGAGRGYGQGAGSAASSVSSASSRSYDYSRRNVRKNCGIPRRQLVVKFRALPCVNCHHHHHH

SEQ ID NO: 10 - DNA, 1590 bp, Artificial
  chimeric protein
atgagagtcaaaacctttgtgatcttgtgctgcgctctgcagtatgtcgcttatacaaatgcaaacatcaatgattttgatgaggactattttgggagtgatgtcactgtccaaagtagtaatacaacagatgaaataattagagatgcatctggggcagttatcgaagaacaaattacaactaaaaaaatgcaacggaaaaataaaaaccatggaatacttggaaaaaatgaaaaaatgatcaagacgttcgttataaccacggattccgacggtaacgagtccattgtagaggaagatgtgctcatgaagacactttccgatggtactgttgctcaaagttatgttgctgctgatgcgggagcatattctcagagcgggccatacgtatcaaacagtggatacagcactcatcaaggatatacgagcgatttcagcactagtgctgcagtcggtgcaggatctatagcagccagtgtaggtgcgggcgttggagcagcttccgttgctggtgcaggaacaggagctggctcaggtgcagctggtggagcaggagcaggtgctgacgctggcgctgcagccgccgctgcggcagcagcacaagcagcagccgcagatgctgccgccgcaggtagtggcgctggtgctggacgagtcggagcttacggaccctacggaggtttagcaagcgctggtgctggtggtgctggcggagccggtggtgcaggtggatacagtggtgcaagtgtcgtctacgtaagtgctggaggagccggagcaggtgccggttcaggcgccggtgctggatcgggtgccggagcaggagctggatcaggtgcaggagcaggtggagcaggagccgcagccggagctggtgctggtgctggttcaggtgcaggatccggttcaggtgcgggcgctggagcaggttccggagcaggagcaggttccggtgctggtgcaggagcaggagctggttcaggtgcagcaggtggagcaggagctggcgctggcgctggcgctgcagccgcagccgcagcagcagcagaagcggcagccgcagctgctgccgccgctgccgccgcaggtagtggagcaggcgctggaggagccggaggctacggagcgggagctggagcaggtgccggtgcaggtgctggcggcgcatctggaggctacggttcttacggatcgggagttgcagcaggtgccggtgcaggagctggtgttggtggtagcaggggagcaggtgttggcgctggtgttggtgctggttatggctccgcattgaattcaggagccggtgccggagcaggtgctggtgctggagctggtggtgctgcaggagctggtgctggtgcaggagcaggagctggcgctggagctggagtcgacagcgtcagttacggagctggcaggggatacggacaaggtgcaggaagtgcagcttcctctgtgtcatctgcttcatctcgcagttacgactattctcgtcgtaacgtccgcaaaaactgtggaattcctagaagacaactagttgttaaattcagagcactgccttgtgtgaattgccatcaccaccatcaccac

SEQ ID NO: 11 - protein, 19 aa, Bombyx mori
  signal peptide of serisin 1
MRFVLCCTLIALAALSVKA

SEQ ID NO: 12 - DNA, 57 bp, Bombyx mori
  nucleic acid sequence coding signal peptide of sericin 1
atgcgtttcgttctgtgctgcactttgattgcgttggctgcgctcagcgtaaaagct

SEQ ID NO: 13 - protein, 18 aa, Bombyx mori
  signal peptide of sericin 2
MKIPYVLLFLVGVAVVNA

SEQ ID NO: 14 - DNA, 54 bp, Bombyx mori
  nucleic acid sequence coding signal peptide of sericin 2
atgaagatcccatacgtcttgctgttccttgtgggcgtggctgtggtcaacgca

SEQ ID NO: 15 - protein, 18 aa, Bombyx mori
  signal peptide of sericin 3
MNCKVALFLIVAIVAVQA

SEQ ID NO: 16 - DNA, 54 bp, Bombyx mori
  nucleic acid sequence coding signal peptide of sericin 3
atgaattgtaaagttgctctattcctgatagtggctattgtagccgtccaggct

SEQ ID NO: 17 - DNA, 870 bp, Bombyx mori
  fibroin H chain promoter
acaaaactgccacacgcatttttttctccactgtaggttgtagttacgcgaaaacaaaatcgttctgtgaaaattcaaacaaaaatattttttcgtaaaaacacttatcaatgagtaaagtaacaattcatgaataatttcatgtaaaaaaaaaatactagaaaaggaatttttcattacgagatgcttaaaaatctgtttcaaggtagagatttttcgatatttcggaaaattttgtaaaactgtaaatccgtaaaattttgctaaacatatattgtgttgttttggtaagtattgacccaagctatcacctcctgcagtatgtcgtgctaattactggacacattgtataacagttccactgtattgacaataataaaacctcttcattgacttgagaatgtctggacagatttggctttgtatttttgatttacaaatgtttttttggtgatttacccatccaaggcattctccaggatggttgtggcatcacgccgattggcaaacaaaaactaaaatgaaactaaaaagaaacagtttccgctgtcccgttcctctagtgggagaaagcatgaagtaagttctttaaatattacaaaaaaattgaacgatattataaaattctttaaaatattaaaagtaagaacaataagatcaattaaatcataattaatcacattgttcatgatcacaatttaatttacttcatacgttgtattgttatgttaaataaaaagattaatttctatgtaattgtatctgtacaatacaatgtgtagatgtttattctatcgaaagtaaatacgtcaaaactcgaaaattttcagtataaaaaggttcaactttttcaaatcagcatcagttcgg

SEQ ID NO: 18 - DNA, 1110 bp, Antheraea pernyi
  fibroin H chain promoter
tccagcgttaccaatgagagcgcttcaaaattctttacaacttcattagaatacgtcgatttttctctacttcatataaatattctatagatgtgtttgctataacataaatacttttaaaaaaatgtctcaacggttgtgaaaactgtcaaaatctgttgcgtagttcagaaaaactaaggaaacatacagaaaatttattttacaaaagtacggagatatataaaaatatttcgattactttagaattacaataaaactatttgacaatttgattgcaaatatagaccatgacaacaccacatctttgttatctaaaacacgtagcgacaacactccttgaacgttgttcgaggattactacgataattggcggttttttttccgcaccgcaagaaaagagtagaaatgtaccgtatttaaatccagtgcggaaattttcacgcagaatgcgtttccatacaattctataggttacatatcttgcggaaataaattcgtgccaaaaagccgaagtgcggggactaataaagattttatttggcattccttctaacctttagatataaatttctgtacgcgcgtatgtcactgaactccccctaaacggctggactaattttgatgaaatattgtttgtgtgttctagtggatccgagaattgtttaaattcgcaaatccggtaggtgaacccgcggttgacttttagattttttttattatcaacaacaacgtccgcccggcccgctagttatgtatgtatttgtaaatgtaatctcaaaccgttcctgttggatcgacatttaatatgtttaagtgaattaattaacgtataacagtcataagaaaatattgcaataaaatcccatcatttattctttagagacaatataaccaaacaacaataagaatcagaatgtaattactctacattgttcatgataggggtttaactatgatattgttttaattctataggattcattactttatcattttgtcaatatttaaaattgtttatttgaaatagttaacgacattacaaagttttcgtataaaagggcgccaaagtctggtctcattatcagttcggttccagctctcataacc

SEQ ID NO: 19 - DNA, 634 bp, Bombyx mori
  fibroin L chain promoter
ggtacggttcgtaaagttcacctgcggctatattcagactcgccaagttacgtcagtcgtattgtaatgagcgatttagtgggcaacttcattctgttaattttgtgtcacggtgcgcgcgcatcgtaaaatttcactctcatagatttttcataacgtgcctaaagaagtataacttcaataatttaaattaaaaaaaaacatgcatagaataattatatgaattatttaaaatgtcatttaccgacattgacataacagacgacgttaacactacaaaacattttaattccacattgctacatattcaacagttaaatttgcgttaattctcgatgcgaacaaatataagaacaatcggatcaattagatcgctttgtttcgagcaacacttagtttaactagaggcgtacacctcaagaaatcatcttcattagaaactaaaccttaaaatcgcattaataaagcatagtcaattttaactgaaatgcaaaatcttttgaacgttagatgctgtcagcgttcgttggtacagttgtttgatatttattttaattgtctttttatatataaatagtggaacattaatcacggaatcctgtatagtatataccgattggtcacataacagacc

SEQ ID NO: 20 - DNA, 1110 bp, Antheraea pernyi; identical to SEQ ID NO: 18
  fibroin L chain promoter

SEQ ID NO: 21 - DNA, 1344 bp, Bombyx mori
  p25 promoter
aagcttagataattcggcattgtgcgccactgagtcgcattatgctctgtaattggaaactaccaaacattgtgtaccctttaatgatattctaatctatatatataaaaatgaattgctgttcgttagtctcgctaaaactcgagaacggccggaccgatttggctaattttggtcttgaattatttgtggaagtccagagaagatttagaaggtttaaataaatatgaaaatgctcggaattaaataaaaataacaattttgttttttctttgatgtgttcccgtcggacggattcctttagtcttttatttatcgactagcgacccgccgcttcgcttcggaaacattaaaatacacatgataccaaaaaaattaaataatttttttttaaaaaaagtagcctatgttcatcaggtacaatgtcggcttctaatggaaaaagaatttttcaaatcggtccagtagtttcggagcctattcgaaacaaacaaacaaacaaatctttcctctttataatattagtatagatagtatagattgaggcactacgaagtctgccgggtcagctagtatactcataaataaggtcgacatctgttgatgatggtgatatcttcaaaattaccttagcgcaatgtagacttatacagtatttctgttttcctaagttaattaccgctgtagccaataccgtctttaccataagcgcacacggggcccggtccagggccgagtgtcgtcgagggggcccgaaagaccggcaagttctctcacacgtttattcccaaaacatttttgtcgggcacattacactttttccacaaatccgtaatcagaaggtatttagcaaggcatatactatgcctataatagaagattttgctcaacagaaatcccgagagaaaccgttatcgaaatcgtaaccaaaaaaccagcagcattctaatatcattaatgacatattatatcatactgtatttgattacctataataaagggtcatactcagtaaaaaaatgttaatataattcgctttttttactttccaaaagggcctcaaattcttgtgtgtccaagggccccatcttagtttaagacgtccctggctgtagcccagttactgccacacaaacatgcttaactcgcgccgcctacgtcgaggagaacattttgcgccttagaaaataaaatggcgtcgccgcggcgcaacaataagaacttaattcgtgcaattgtttccacgacgctatttatttaacgttattcgttgtgaggaacaatactttgtataattaatgttgatcagtgcctaacgacgcagttgtttattattcgcgcaac

SEQ ID NO: 22 - DNA, 244 bp, Bombyx mori
  hsp70 terminator
aatgaatcgtagatactgaaaaaccccgcaagttcacttcaactgtgcatcgtgcaccatctcaatttctttcatttatacatcgttttgccttcttttatgtaactatactcctctaagtttcaatcttggccatgtaacctctgatctatagaattttttaaatgactagaattaatgcccatcttttttttggacctaaattcttcatgaaaatatattacgagggcttattcagaagctt

SEQ ID NO: 23 - DNA, 207 bp, SV40 virus
  SV40 terminator
tcagccataccacatttgtagaggttttacttgctttaaaaaacctcccacacctccccctgaacctgaaacataaaatgaatgcaattgttgttgttaacttgtttattgcagcttataatggttacaaataaagcaatagcatcacaaatttcacaaataaagcatttttttcactgcattctagttgtggtttgtccaaactca

SEQ ID NO: 24 - DNA, 765 bp, Eumeta japonica
atgagagctctgaccttcgtgatcctgtgctgcgctttgcagcaatatgcatcagcaaaggcggattggtatgaagattggaaaaaaaaccaaggttcatttagagaaacagacttagcagacactgacgaatatcaaacagatagtaatggtacaatgtttgaaaaaaaaacaacaagaaaaaagttcgaaaaagatggaagtactatggtaaacagtgattccggagaagataaaattgtacgaactttcgtcgtggaaactgacgcatcaggacatgaagttatttatgaagaagatgtagtcattaaaaaagttccaggtaaacggaagaaagtttcacaggcaaatgctaaagctagtgctatagcagccagtgtaggtgcgggcgttggagcagcttccgttgctggtgcaggaacaggagctggctcaggtgcagctggtggagcaggagcaggtgctgacgctggcgctgcagccgccgctgcggcagcagcacaagcagcagccgcagctgctgccgccgcaggtagtggcgctggtgctggacgagtcggagcttacggaccctacggaggtttagcaagcgctggtgctggtggtgctggcggagccggtggtgcaggtggatacggtggtgcaagtgtcgtctacgtaggtggcggaggagccggagcaggtgccggttcaggcgccggtgctggatcgggtgccggagcaggagctggatcaggtgcaggagcaggtggagcaggagccgca

SEQ ID NO: 25 - DNA, 1023 bp, Eumeta japonica
gcaggtgctggcggcgctgctggtgctggtggtgctggcggagccggtggtgcaggtggatacggtggtgcaggtgtcgtctacgtaagtgctggaggagccggagcaggtgccggttcaggcgccggtgctggatcgggtgccggagcaggagctggatcaggtgcaggagcaggtggagcaggagccgcagccggagctggtgctggtgctggttcaggtgcaggatccggttcaggtgcgggcgctggagcaggttccggagcaggagcaggttccggtgctggtgcaggagcaggagctggttcaggtgcagcaggtggagcaggagctggcgctggcgctggcgctgcagccgcagccgcagcagcagcagaagcggcagccgcagctgccgccgccgctgccgccgcaggtagtggagcaggcgctggaggagccggaggctacggagcgggagctggagcaggtgccggtgcaggtgctggcggcgcatctggaggctacggttcttacggatcgggagttgcagcaggtgccggtgcaggagctggtgttggtggtagcaggggagcaggtgttggcgctggtgttggtgctggttatggctccgcattgaattcaggagccggtgccggagcaggtgctggtgctggagctggtggtgctgcaggagctggtgctggtgcaggagcaggagctggttcaggtgcagcaggtggagcaggagctggcgctggcgctggcgctgcagccgcagccgcagcagcagcagaagcggcagccgcagctgccgccgccgctgccgccgctggaggagccggaggctacggagcgggagctggagcaggtgccggtgcaggtgctggcggcgctggtggtgctggtggtgctggcggagccggtggtgcaggtggatacggtggtgcaggtgtcgtctacgtaagtgctggaggagccggagcaggtgccggttcaggcgccggtgctggatcgggtgccggagcaggagctggatcaggt

SEQ ID NO: 26 - DNA, 333 bp, Eumeta japonica
ggtgctggcggcgcatctggaggctacggttcttacggatcgggagttgcagcaggtgccggtgcaggagctggtgttggtggtagcaggggagcaggtgttggcgctggtgttggtgctggttatggctccgcattgaattcaggagccggtgccggagcaggtgctggtgctggagctggtggtgctgcaggagctggtgctggtgcaggagcaggagctggcgctggagctggattcgcttcttatggaagaccaggtgttcgtggatgtcaactgtctcgtaaataccttttggttaaagttggtttaagatccacatgctcagattgt

SEQ ID NO: 27 - DNA, 29 bp, Artificial
  EvHFB-F21 primer
catcagcaaaggcggattggtatgaagat

SEQ ID NO: 28 - DNA, 29 bp, Artificial
  EvHFB-R26 primer
ggctcctccagcacttacgtagacgacac

SEQ ID NO: 29 - DNA, 26 bp, Artificial
  EvHFB-F26 primer
tgtcgtctacgtaggtggcggaggag

SEQ ID NO: 30 - DNA, 30 bp, Artificial
  EvHFB-R12 primer
atttacgagacagttgacatccacgaacac

SEQ ID NO: 31 - DNA, 25 bp, Artificial
  EvHFB-F12 primer
cagcaaaggcggattggtatgaaga

SEQ ID NO: 32 - DNA, 32 bp, Artificial
  EvHFB-F31 primer
gctagatctatagcagccagtgtaggtgcggg

SEQ ID NO: 33 - DNA, 33 bp, Artificial
  EvHFB-R31 primer
cctggtcttccataagagtcgactccagctcca